European Patent Application EP 4 434 541 A2, published September 25, 2024. Title: ANTIBODIES SPECIFIC TO DELTA 1 CHAIN OF T CELL RECEPTOR. Applicant: NEW YORK UNIVERSITY. Application EP. The sequence listing filed with the application follows.

SEQUENCE LISTING (94 sequences)

SEQ ID NO: 1 - protein, 130 aa, Homo sapiens
EVQLVESGGGLVQPGGSLRLSCAASGFTVSSSSIHWVRQAPGKGLEWVASIYSSSGYTYYADSVKGRFTISADTSKNTAYLQMNSLRAEDTAVYYCARDPGMYYWYYSGSAYEGYGLDYWGQGTLVTVSS

SEQ ID NO: 2 - protein, 108 aa, Homo sapiens
DIQMTQSPSSLSASVGDRVTITCRASQSVSSAVAWYQQKPGKAPKLLIYSASSLYSGVPSRFSGSRSGTDFTLTISSLQPEDFATYYCQQSGDDLITFGQGTKVEIKR

SEQ ID NO: 3 - protein, 130 aa, Homo sapiens
EVQLVESGGGLVQPGGSLRLSCAASGFTVSSSSIHWVRQAPGKGLEWVASIYSSSGYTYYADSVKGRFTISADTSKNTAYLQMNSLRAEDTAVYYCARDPGSYYWYYSGSAYEGYGLDYWGQGTLVTVSS

SEQ ID NO: 4 - protein, 110 aa, Homo sapiens
DIQMTQSPSSLSASVGDRVTITCRASQSVSSAVAWYQQKPGKAPKLLIYAASSLQSGVPSRFSGSRSGTDFTLTISSLQPEDFATYYCQQRSRVYSLVTFGQGTKVEIKR

SEQ ID NO: 5 - protein, 110 aa, Homo sapiens
DIQMTQSPSSLSASVGDRVTITCRASQSVSSAVAWYQQKPGKAPKLLIYAASSLQSGVPSRFSGSRSGTDFTLTISSLQPEDFATYYCQQMDRFYSLITFGQGTKVEIKR

SEQ ID NO: 6 - protein, 110 aa, Homo sapiens
DIQMTQSPSSLSASVGDRVTITCRASQSVSSAVAWYQQKPGKAPKLLIYAASSLQSGVPSRFSGSRSGTDFTLTISSLQPEDFATYYCQQYCRKSSLFTFGQGTKVEIKR

SEQ ID NO: 7 - protein, 110 aa, Homo sapiens
DIQMTQSPSSLSASVGDRVTITCRASQSVSSAVAWYQQKPGKAPKLLIYAASSLQSGVPSRFSGSRSGTDFTLTISSLQPEDFATYYCQQQQRTSYLITFGQGTKVEIKR

SEQ ID NO: 8 - protein, 110 aa, Homo sapiens
DIQMTQSPSSLSASVGDRVTITCRASQSVSSAVAWYQQKPGKAPKLLIYAASSLQSGVPSRFSGSRSGTDFTLTISSLQPEDFATYYCQQRSRYYSLITFGQGTKVEIKR

SEQ ID NO: 9 - protein, 110 aa, Homo sapiens
DIQMTQSPSSLSASVGDRVTITCRASQSVSSAVAWYQQKPGKAPKLLIYAASSLQSGVPSRFSGSRSGTDFTLTISSLQPEDFATYYCQQQSKYPFLITFGQGTKVEIKR

SEQ ID NO: 10 - protein, 110 aa, Homo sapiens
DIQMTQSPSSLSASVGDRVTITCRASQSVSSAVAWYQQKPGKAPKLLIYAASSLQSGVPSRFSGSRSGTDFTLTISSLQPEDFATYYCQQSNRSYPPLTFGQGTKVEIKR

SEQ ID NO: 11 - protein, 110 aa, Homo sapiens
DIQMTQSPSSLSASVGDRVTITCRASQSVSSAVAWYQQKPGKAPKLLIYAASSLQSGVPSRFSGSRSGTDFTLTISSLQPEDFATYYCQQIGRRSSLITFGQGTKVEIKR

SEQ ID NO: 12 - protein, 110 aa, Homo sapiens
DIQMTQSPSSLSASVGDRVTITCRASQSVSSAVAWYQQKPGKAPKLLIYAASSLQSGVPSRFSGSRSGTDFTLTISSLQPEDFATYYCQQQQRYSYLITFGQGTKVEIKR

SEQ ID NO: 13 - protein, 110 aa, Homo sapiens
DIQMTQSPSSLSASVGDRVTITCRASQSVSSAVAWYQQKPGKAPKLLIYAASSLQSGVPSRFSGSRSGTDFTLTISSLQPEDFATYYCQQSSRNSKLITFGQGTKVEIKR

SEQ ID NO: 14 - protein, 110 aa, Homo sapiens
DIQMTQSPSSLSASVGDRVTITCRASQSVSSAVAWYQQKPGKAPKLLIYAASSLQSGVPSRFSGSRSGTDFTLTISSLQPEDFATYYCQQWMRSSSLFTFGQGTKVEIKR

SEQ ID NO: 15 - protein, 108 aa, Homo sapiens
DIQMTQSPSSLSASVGDRVTITCRASQSVSSAVAWYQQKPGKAPKLLIYAASSLQSGVPSRFSGSRSGTDFTLTISSLQPEDFATYYCQQSGDDLITFGQGTKVEIKR

SEQ ID NO: 16 - protein, 110 aa, Homo sapiens
DIQMTQSPSSLSASVGDRVTITCRASQSVSSAVAWYQQKPGKAPKLLIYAASSLQSGVPSRFSGSRSGTDFTLTISSLQPEDFATYYCQQQTSWPYLITFGQGTKVEIKR

SEQ ID NO: 17 - protein, 130 aa, Homo sapiens
EVQLVESGGGLVQPGGSLRLSCAASGFTFSSSDIHWVRQAPGKGLEWVASIYSSSGYTYYADSVKGRFTISADTSKNTAYLQMNSLRAEDTAVYYCARDPGSYYWYYSGSAYEGYGLDYWGQGTLVTVSS

SEQ ID NO: 18 - protein, 130 aa, Homo sapiens
EVQLVESGGGLVQPGGSLRLSCAASGFTFSSSSIHWVRQAPGKGLEWVASIYSSSGYTYYADSVKGRFTISADTSKNTAYLQMNSLRAEDTAVYYCARDPGSYYWYYSGSAYEGYGLDYWGQGTLVTVSS

SEQ ID NO: 19 - protein, 130 aa, Homo sapiens
EVQLVESGGGLVQPGGSLRLSCAASGFTFSGTDIHWVRQAPGKGLEWVASIYSSSGYTYYADSVKGRFTISADTSKNTAYLQMNSLRAEDTAVYYCARDPGSYYWYYSGSAYEGYGLDYWGQGTLVTVSS

SEQ ID NO: 20 - protein, 130 aa, Homo sapiens
EVQLVESGGGLVQPGGSLRLSCAASGFTFSASSIHWVRQAPGKGLEWVASIYSSSGYTYYADSVKGRFTISADTSKNTAYLQMNSLRAEDTAVYYCARDPGSYYWYYSGSAYEGYGLDYWGQGTLVTVSS

SEQ ID NO: 21 - protein, 130 aa, Homo sapiens
EVQLVESGGGLVQPGGSLRLSCAASGFTFSSNDIHWVRQAPGKGLEWVASIYSSSGYTYYADSVKGRFTISADTSKNTAYLQMNSLRAEDTAVYYCARDPGSYYWYYSGSAYEGYGLDYWGQGTLVTVSS

SEQ ID NO: 22 - protein, 130 aa, Homo sapiens
EVQLVESGGGLVQPGGSLRLSCAASGFTFTGSSIHWVRQAPGKGLEWVASIYSSSGYTYYADSVKGRFTISADTSKNTAYLQMNSLRAEDTAVYYCARDPGSYYWYYSGSAYEGYGLDYWGQGTLVTVSS

SEQ ID NO: 23 - protein, 130 aa, Homo sapiens
EVQLVESGGGLVQPGGSLRLSCAASGFTFTSSDIHWVRQAPGKGLEWVASIYSSSGYTYYADSVKGRFTISADTSKNTAYLQMNSLRAEDTAVYYCARDPGSYYWYYSGSAYEGYGLDYWGQGTLVTVSS

SEQ ID NO: 24 - protein, 130 aa, Homo sapiens
EVQLVESGGGLVQPGGSLRLSCAASGFTFTANDIHWVRQAPGKGLEWVASIYSSSGYTYYADSVKGRFTISADTSKNTAYLQMNSLRAEDTAVYYCARDPGSYYWYYSGSAYEGYGLDYWGQGTLVTVSS

SEQ ID NO: 25 - protein, 130 aa, Homo sapiens
EVQLVESGGGLVQPGGSLRLSCAASGFTFTSSSIHWVRQAPGKGLEWVASIYSSSGYTYYADSVKGRFTISADTSKNTAYLQMNSLRAEDTAVYYCARDPGSYYWYYSGSAYEGYGLDYWGQGTLVTVSS

SEQ ID NO: 26 - protein, 233 aa, Homo sapiens
AQKVTQAQSSVSMPVRKAVTLNCLYETSWWSYYIFWYKQLPSKEMIFLIRQGSDEQNAKSGRYSVNFKKAAKSVALTISALQLEDSAKYFCALGVYAHSLTGGYRGGADKLIFGKGTRVTVEPRSQPHTKPSVFVMKNGTNVACLVKEFYPKDIRINLVSSKKITEFDPAIVISPSGKYNAVKLGKYEDSNSVTCSVQHDNKTVHSTDFEVKTDSTDHVKPKETENTKQPSKS

SEQ ID NO: 27 - protein, 234 aa, Homo sapiens
AQKVTQAQSSVSMPVRKAVTLNCLYETSWWSYYIFWYKQLPSKEMIFLIRQGSDEQNAKSGRYSVNFKKAAKSVALTISALQLEDSAKYFCALGPRPSYSEELGDTHRADKLIFGKGTRVTVEPRSQPHTKPSVFVMKNGTNVACLVKEFYPKDIRINLVSSKKITEFDPAIVISPSGKYNAVKLGKYEDSNSVTCSVQHDNKTVHSTDFEVKTDSTDHVKPKETENTKQPSKS

SEQ ID NO: 28 - protein, 227 aa, Homo sapiens
AQKVTQAQSSVSMPVRKAVTLNCLYETSWWSYYIFWYKQLPSKEMIFLIRQGSDEQNAKSGRYSVNFKKAAKSVALTISALQLEDSAKYFCALGEPNHFLNTDKLIFGKGTRVTVEPRSQPHTKPSVFVMKNGTNVACLVKEFYPKDIRINLVSSKKITEFDPAIVISPSGKYNAVKLGKYEDSNSVTCSVQHDNKTVHSTDFEVKTDSTDHVKPKETENTKQPSKS

SEQ ID NO: 29 - protein, 229 aa, Homo sapiens
AIELVPEHQTVPVSIGVPATLRCSMKGEAIGNYYINWYRKTQGNTMTFIYREKDIYGPGFKDNFQGDIDIAKNLAVLKILAPSERDEGSYYCACDTLGMGGEYTDKLIFGKGTRVTVEPRSQPHTKPSVFVMKNGTNVACLVKEFYPKDIRINLVSSKKITEFDPAIVISPSGKYNAVKLGKYEDSNSVTCSVQHDNKTVHSTDFEVKTDSTDHVKPKETENTKQPSKS

SEQ ID NO: 30 - protein, 242 aa, Homo sapiens
AGHLEQPQISSTKTLSKTARLECVVSGITISATSVYWYRERPGEVIQFLVSISYDGTVRKESGIPSGKFEVDRIPETSTSTLTIHNVEKQDIATYYCALWEAQQELGKKIKVFGPGTKLIITDKQLDADVSPKPTIFLPSIAETKLQKAGTYLCLLEKFFPDVIKIHWEEKKSNTILGSQEGNTMKTNDTYMKFSWLTVPEKSLDKEHRCIVRHENNKNGVDQEIIFPPIKTDVITMDPKDN

SEQ ID NO: 31 - protein, 330 aa, Homo sapiens
ASTKGPSVFPLAPSSKSTSGGTAALGCLVKDYFPEPVTVSWNSGALTSGVHTFPAVLQSSGLYSLSSVVTVPSSSLGTQTYICNVNHKPSNTKVDKKVEPKSCDKTHTCPPCPAPELLGGPSVFLFPPKPKDTLMISRTPEVTCVVVDVSHEDPEVKFNWYVDGVEVHNAKTKPREEQYNSTYRVVSVLTVLHQDWLNGKEYKCKVSNKALPAPIEKTISKAKGQPREPQVYTLPPSREEMTKNQVSLTCLVKGFYPSDIAVEWESNGQPENNYKTTPPVLDSDGSFFLYSKLTVDKSRWQQGNVFSCSVMHEALHNHYTQKSLSLSPGK

SEQ ID NO: 32 - protein, 223 aa, Macaca fascicularis
AQKVTQAQSSVSMPVEKAVTLNCQYETSSWSYDLFWYKQLPGKEMIFLIRQGSSEQNARDGRYSVNFKKEASFIALTISALQLEDSATYFCALRRPFTAQLFFGKGTQLIVEPERQPHTKPSVFVMKNGTNVACLVKDFYPKDIRINLESSKKITEFDPAIVVSPSGKYNAVKLGQYADSNSVTCSVQHNKEVVYSTDFEVKTNSTDHLKPTETENTKQPSKS

SEQ ID NO: 33 - protein, 235 aa, Macaca fascicularis
AQKVTQAQSSVSMPVGKAVTLNCQYETSSWSYYLFWYKQLPGKEMIFLIHQGSSQQNARNGRYSVNFQKAASSITLTISALQLEDSATYFCALRERPPNPGPFVLGVYATAQLFFGKGTQLIVEPERQPHTKPSVFVMKNGTNVACLVKDFYPKDIRINLESSKKITEFDPAIVVSPSGKYNAVKLGQYADSNSVTCSVQHNKEVVYSTDFEVKTNSTDHLKPTETENTKQPSKS

SEQ ID NO: 34 - protein, 235 aa, Macaca fascicularis
AQKVTQAQSSVSMPVEKAVTLNCQYETSWWSYDLFWYKQLPGKEMIFLIRQSSSEQNARDGRYSANFKKEASSKSFIALTISALQLEDSATYFCALPLQVRGPTGGIRVYDKLIFGKGTRVTVEPKRQPHTKPSVFVMKNGTNVACLVKDFYPKDIRINLESSKKITEFDPAIVVSPSGKYNAVKLGQYADSNSVTCSVQHNKEVVYSTDFEVKTNSTDHLKPTETENTKQPSKS

SEQ ID NO: 35 - protein, 227 aa, Homo sapiens
AIELVPEHQTVPVSIGVPATLRCSMKGEAIGNYYINWYRKTQGNTMTFIYREKDIYGPGFKDNFQGDIDIAKNLAVLKILAPSERDEGSYYCACDTSSSSGTDKLIFGKGTRVTVEPRSQPHTKPSVFVMKNGTNVACLVKEFYPKDIRINLVSSKKITEFDPAIVISPSGKYNAVKLGKYEDSNSVTCSVQHDNKTVHSTDFEVKTDSTDHVKPKETENTKQPSKS

SEQ ID NO: 36 - protein, 228 aa, Homo sapiens
AIELVPEHQTVPVSIGVPATLRCSMKGEAIGNYYINWYRKTQGNTMTFIYREKDIYGPGFKDNFQGDIDIAKNLAVLKILAPSERDEGSYYCACDILGDKGNTDKLIFGKGTRVTVEPRSQPHTKPSVFVMKNGTNVACLVKEFYPKDIRINLVSSKKITEFDPAIVISPSGKYNAVKLGKYEDSNSVTCSVQHDNKTVHSTDFEVKTDSTDHVKPKETENTKQPSKS

SEQ ID NO: 37 - protein, 229 aa, Macaca fascicularis
AVELVPEHQTVIVSVGDPATLKCSMKGEAISNYYINWYRKTQGNTMTFIYREKGIYGPGFKDNFQGDIDTEENQAVLKILAPSERDEGSYYCASDILSWVDSYTDKLIFGKGTRVTVEPKRQPHTKPSVFVMKNGTNVACLVKDFYGKDIRINLESSKKITEFDPAIVVSPSGKYNAVKLGQYADSNSVTCSVQHNKEVVYSTDFEVKTNSTDHLKPTETENTKQPSKS

SEQ ID NO: 38 - protein, 240 aa, Homo sapiens
SSNLEGRTKSVTRQTGSSAEITCDLTVTNTFYIHWYLHQEGKAPQRLLYYDVSTARDVLESGLSPGKYYTHTPRRWSWILRLQNLIENDSGVYYCATWDRPLNAWIKTFAKGTRLIVTSPDKQLDADVSPKPTIFLPSIAETKLQKAGTYLCLLEKFFPDVIKIHWQEKKSNTILGSQEGNTMKTNDTYMKFSWLTVPEKSLDKEHRCIVRHENNKNGVDQEIIFPPIKTDVITMDPKDN

SEQ ID NO: 39 - protein, 236 aa, Homo sapiens
SSNLEGRTKSVIRQTGSSAEITCDLAEGSTGYIHWYLHQEGKAPQRLLYYDSYTSSVVLESGISPGKYDTYGSTRKNLRMILRNLIENDSGVYYCATWDEKYYKKLFGSGTTLVVTDKQLDADVSPKPTIFLPSIAETKLQKAGTYLCLLEKFFPDVIKIHWQEKKSNTILGSQEGNTMKTNDTYMKFSWLTVPEKSLDKEHRCIVRHENNKNGVDQEIIFPPIKTDVITMDPKDN

SEQ ID NO: 40 - protein, 235 aa, Homo sapiens
SSNLEGGTKSVTRPTRSSAEITCDLTVINAFYIHWYLHQEGKAPQRLLYYDVSNSKDVLESGLSPGKYYTHTPRRWSWILILRNLIENDSGVYYCATWDRLRKKLFGSGTTLVVTDKQLDADVSPKPTIFLPSIAETKLQKAGTYLCLLEKFFPDVIKIHWQEKKSNTILGSQEGNTMKTNDTYMKFSWLTVPEKSLDKEHRCIVRHENNKNGVDQEIIFPPIKTDVITMDPKDN

SEQ ID NO: 41 - protein, 234 aa, Homo sapiens
SSNLEGRTKSVTRPTGSSAVITCDLPVENAVYTHWYLHQEGKAPQRLLYYDSYNSRVVLESGISREKYHTYASTGKSLKFILENLIERDSGVYYCATWDWGKKLFGSGTTLVVTDKQLDADVSPKPTIFLPSIAETKLQKAGTYLCLLEKFFPDVIKIHWQEKKSNTILGSQEGNTMKTNDTYMKFSWLTVPEKSLDKEHRCIVRHENNKNGVDQEIIFPPIKTDVITMDPKDN

SEQ ID NO: 42 - protein, 241 aa, Macaca fascicularis
AGHLEQPQISSTKMLSKTARLECVVSGVTISETSIYWYRERPGEVIQFLVCIFYDGTVKKESSIPSGKFEVDRIPKTSTSTLTIHNVEKQDIATYYCALWEVQQFGRKVKLFGPGTKLIITDKHLDADVSPKPTIFLPSIAETNLHKAGTYLCLLENFFPDVIKIHWQEKKSNTILGSQEGNTVKTNDTYMKFSWLTVPEKSLDKEHRCIVRHENNKNGVDQEIIFPPIKTDVTTMDPKDN

SEQ ID NO: 43 - protein, 130 aa, Homo sapiens
EVQLVESGGGLVQPGGSLRLSCAASGFTFSANDIHWVRQAPGKGLEWVASIYSSSGYTYYADSVKGRFTISADTSKNTAYLQMNSLRAEDTAVYYCARDPGSYYWYYSGSAYEGYGLDYWGQGTLVTVSS

SEQ ID NO: 44 - protein, 130 aa, Homo sapiens
EVQLVESGGGLVQPGGSLRLSCAASGFTFSATDIHWVRQAPGKGLEWVASIYSSSGYTYYADSVKGRFTISADTSKNTAYLQMNSLRAEDTAVYYCARDPGSYYWYYSGSAYEGYGLDYWGQGTLVTVSS

SEQ ID NO: 45 - protein, 130 aa, Homo sapiens
EVQLVESGGGLVQPGGSLRLSCAASGFTFSGSDIHWVRQAPGKGLEWVASIYSSSGYTYYADSVKGRFTISADTSKNTAYLQMNSLRAEDTAVYYCARDPGSYYWYYSGSAYEGYGLDYWGQGTLVTVSS

SEQ ID NO: 46 - protein, 9 aa, Homo sapiens
  SITE 3: note = MISC_FEATURE - X may be F or V
  SITE 4: note = MISC_FEATURE - X may be S or T
  SITE 5: note = MISC_FEATURE - X may be G, A, or S
  SITE 6: note = MISC_FEATURE - X may be T, N, or S
  SITE 7: note = MISC_FEATURE - X may be D or S
FTXXXXXIH

SEQ ID NO: 47 - protein, 451 aa, Homo sapiens
EVQLVESGGGLVQPGGSLRLSCAASGFTVSSSSIHWVRQAPGKGLEWVAYISSSSGYTYYADSVKGRFTISADTSKNTAYLQMNSLRAEDTAVYYCARYWSYPSWWPYRGMDYWGQGTLVTVSSASTKGPSVFPLAPCSRSTSESTAALGCLVKDYFPEPVTVSWNSGALTSGVHTFPAVLQSSGLYSLSSVVTVPSSSLGTKTYTCNVDHKPSNTKVDKRVESKYGPPCPSCPAPEFLGGPSVFLFPPKPKDTLMISRTPEVTCVVVDVSQEDPEVQFNWYVDGVEVHNAKTKPREEQFNSTYRVVSVLTVLHQDWLNGKEYKCKVSNKGLPSSIEKTISKAKGQPREPQVYTLPPSQEEMTKNQVSLTCLVKGFYPSDIAVEWESNGQPENNYKTTPPVLDSDGSFFLYSRLTVDKSRWQEGNVFSCSVMHEALHNHYTQKSLSLSPGK

SEQ ID NO: 48 - protein, 20 aa, Homo sapiens
  SITE 3: note = MISC_FEATURE - X may be S or M
PGXYYWYYSGSAYEGYGLDY

SEQ ID NO: 49 - protein, 457 aa, Homo sapiens
EVQLVESGGGLVQPGGSLRLSCAASGFTFTANDIHWVRQAPGKGLEWVASIYSSSGYTYYADSVKGRFTISADTSKNTAYLQMNSLRAEDTAVYYCARDPGSYYWYYSGSAYEGYGLDYWGQGTLVTVSSASTKGPSVFPLAPCSRSTSESTAALGCLVKDYFPEPVTVSWNSGALTSGVHTFPAVLQSSGLYSLSSVVTVPSSSLGTKTYTCNVDHKPSNTKVDKRVESKYGPPCPPCPAPEFLGGPSVFLFPPKPKDTLMISRTPEVTCVVVDVSQEDPEVQFNWYVDGVEVHNAKTKPREEQFNSTYRVVSVLTVLHQDWLNGKEYKCKVSNKGLPSSIEKTISKAKGQPREPQVYTLPPSQEEMTKNQVSLTCLVKGFYPSDIAVEWESNGQPENNYKTTPPVLDSDGSFFLYSRLTVDKSRWQEGNVFSCSVMHEALHNHYTQKSLSLSLGK

SEQ ID NO: 50 - protein, 7 aa, Homo sapiens
  SITE 1: note = MISC_FEATURE - X may be S or A
  SITE 6: note = MISC_FEATURE - X may be Y or Q
XASSLXS

SEQ ID NO: 51 - protein, 11 aa, Homo sapiens
  SITE 3: note = MISC_FEATURE - X may be S or Q
  SITE 4: note = MISC_FEATURE - X may be G, S, or T
  SITE 5: note = MISC_FEATURE - X may be D, K, or S
  SITE 6: note = MISC_FEATURE - X may be Y, W, or absent
  SITE 7: note = MISC_FEATURE - X may be P or absent
  SITE 8: note = MISC_FEATURE - X may be D, F, or Y
QQXXXXXXLIT

SEQ ID NO: 52 - protein, 9 aa, Homo sapiens
FTVSSSSIH

SEQ ID NO: 53 - protein, 17 aa, Homo sapiens
SIYSSSGYTYYADSVKG

SEQ ID NO: 54 - protein, 21 aa, Homo sapiens
DPGSYYWYYSGSAYEGYGLDY

SEQ ID NO: 55 - protein, 11 aa, Homo sapiens
RASQSVSSAVA

SEQ ID NO: 56 - protein, 7 aa, Homo sapiens
AASSLQS

SEQ ID NO: 57 - protein, 11 aa, Homo sapiens
QQQSKYPFLIT

SEQ ID NO: 58 - protein, 7 aa, Homo sapiens
SASSLYS

SEQ ID NO: 59 - protein, 9 aa, Homo sapiens
QQSGDDLIT

SEQ ID NO: 60 - protein, 11 aa, Homo sapiens
QQQTSWPYLIT

SEQ ID NO: 61 - protein, 9 aa, Homo sapiens
FTFSSSDIH

SEQ ID NO: 62 - protein, 9 aa, Homo sapiens
FTFSSSSIH

SEQ ID NO: 63 - protein, 9 aa, Homo sapiens
FTFSGTDIH

SEQ ID NO: 64 - protein, 9 aa, Homo sapiens
FTFSASSIH

SEQ ID NO: 65 - protein, 9 aa, Homo sapiens
FTFSSNDIH

SEQ ID NO: 66 - protein, 9 aa, Homo sapiens
FTFTGSSIH

SEQ ID NO: 67 - protein, 9 aa, Homo sapiens
FTFTSSDIH

SEQ ID NO: 68 - protein, 9 aa, Homo sapiens
FTFTANDIH

SEQ ID NO: 69 - protein, 9 aa, Homo sapiens
FTFTSSSIH

SEQ ID NO: 70 - protein, 9 aa, Homo sapiens
FTFSANDIH

SEQ ID NO: 71 - protein, 9 aa, Homo sapiens
FTFSATDIH

SEQ ID NO: 72 - protein, 9 aa, Homo sapiens
FTFSGSDIH

SEQ ID NO: 73 - protein, 106 aa, Homo sapiens
TVAAPSVFIFPPSDEQLKSGTASVVCLLNNFYPREAKVQWKVDNALQSGNSQESVTEQDSKDSTYSLSSTLTLSKADYEKHKVYACEVTHQGLSSPVTKSFNRGEC

SEQ ID NO: 74 - protein, 330 aa, Homo sapiens
ASTKGPSVFPLAPSSKSTSGGTAALGCLVKDYFPEPVTVSWNSGALTSGVHTFPAVLQSSGLYSLSSVVTVPSSSLGTQTYICNVNHKPSNTKVDKKVEPKSCDKTHTCPPCPAPEAAGGPSVFLFPPKPKDTLMISRTPEVTCVVVDVSHEDPEVKFNWYVDGVEVHNAKTKPREEQYNSTYRVVSVLTVLHQDWLNGKEYKCKVSNKALGAPIEKTISKAKGQPREPQVYTLPPSREEMTKNQVSLTCLVKGFYPSDIAVEWESNGQPENNYKTTPPVLDSDGSFFLYSKLTVDKSRWQQGNVFSCSVMHEALHNHYTQKSLSLSPGK

SEQ ID NO: 75 - protein, 327 aa, Homo sapiens
ASTKGPSVFPLAPCSRSTSESTAALGCLVKDYFPEPVTVSWNSGALTSGVHTFPAVLQSSGLYSLSSVVTVPSSSLGTKTYTCNVDHKPSNTKVDKRVESKYGPPCPSCPAPEFLGGPSVFLFPPKPKDTLMISRTPEVTCVVVDVSQEDPEVQFNWYVDGVEVHNAKTKPREEQFNSTYRVVSVLTVLHQDWLNGKEYKCKVSNKGLPSSIEKTISKAKGQPREPQVYTLPPSQEEMTKNQVSLTCLVKGFYPSDIAVEWESNGQPENNYKTTPPVLDSDGSFFLYSRLTVDKSRWQEGNVFSCSVMHEALHNHYTQKSLSLSLGK

SEQ ID NO: 76 - protein, 327 aa, Homo sapiens
ASTKGPSVFPLAPCSRSTSESTAALGCLVKDYFPEPVTVSWNSGALTSGVHTFPAVLQSSGLYSLSSVVTVPSSSLGTKTYTCNVDHKPSNTKVDKRVESKYGPPCPPCPAPEFLGGPSVFLFPPKPKDTLMISRTPEVTCVVVDVSQEDPEVQFNWYVDGVEVHNAKTKPREEQFNSTYRVVSVLTVLHQDWLNGKEYKCKVSNKGLPSSIEKTISKAKGQPREPQVYTLPPSQEEMTKNQVSLTCLVKGFYPSDIAVEWESNGQPENNYKTTPPVLDSDGSFFLYSRLTVDKSRWQEGNVFSCSVMHEALHNHYTQKSLSLSLGK

SEQ ID NO: 77 - protein, 327 aa, Homo sapiens
ASTKGPSVFPLAPCSRSTSESTAALGCLVKDYFPEPVTVSWNSGALTSGVHTFPAVLQSSGLYSLSSVVTVPSSSLGTKTYTCNVDHKPSNTKVDKRVESKYGPPCPPCPAPEFLGGPSVFLFPPKPKDTLMISRTPEVTCVVVDVSQEDPEVQFNWYVDGVEVHNAKTKPREEQFNSTYRVVSVLTVLHQDWLNGKEYKCKVSNKGLPSSIEKTISKAKGQPREPQVYTLPPSQEEMTKNQVSLTCLVKGFYPSDIAVEWESNGQPENNYKTTPPVLDSDGSFFLYSRLTVDKSRWQEGNVFSCSVMHEALHNHYTQKSLSLSPGK

SEQ ID NO: 78 - protein, 216 aa, Homo sapiens
DIQMTQSPSSLSASVGDRVTITCRASQSVSSAVAWYQQKPGKAPKLLIYAASSLQSGVPSRFSGSRSGTDFTLTISSLQPEDFATYYCQQQSKYPFLITFGQGTKVEIKRTVAAPSVFIFPPSDEQLKSGTASVVCLLNNFYPREAKVQWKVDNALQSGNSQESVTEQDSKDSTYSLSSTLTLSKADYEKHKVYACEVTHQGLSSPVTKSFNRGEC

SEQ ID NO: 79 - protein, 460 aa, Homo sapiens
EVQLVESGGGLVQPGGSLRLSCAASGFTFTANDIHWVRQAPGKGLEWVASIYSSSGYTYYADSVKGRFTISADTSKNTAYLQMNSLRAEDTAVYYCARDPGSYYWYYSGSAYEGYGLDYWGQGTLVTVSSASTKGPSVFPLAPSSKSTSGGTAALGCLVKDYFPEPVTVSWNSGALTSGVHTFPAVLQSSGLYSLSSVVTVPSSSLGTQTYICNVNHKPSNTKVDKKVEPKSCDKTHTCPPCPAPELLGGPSVFLFPPKPKDTLMISRTPEVTCVVVDVSHEDPEVKFNWYVDGVEVHNAKTKPREEQYNSTYRVVSVLTVLHQDWLNGKEYKCKVSNKALPAPIEKTISKAKGQPREPQVYTLPPSREEMTKNQVSLTCLVKGFYPSDIAVEWESNGQPENNYKTTPPVLDSDGSFFLYSKLTVDKSRWQQGNVFSCSVMHEALHNHYTQKSLSLSPGK

SEQ ID NO: 80 - protein, 457 aa, Homo sapiens
EVQLVESGGGLVQPGGSLRLSCAASGFTFTANDIHWVRQAPGKGLEWVASIYSSSGYTYYADSVKGRFTISADTSKNTAYLQMNSLRAEDTAVYYCARDPGSYYWYYSGSAYEGYGLDYWGQGTLVTVSSASTKGPSVFPLAPCSRSTSESTAALGCLVKDYFPEPVTVSWNSGALTSGVHTFPAVLQSSGLYSLSSVVTVPSSSLGTKTYTCNVDHKPSNTKVDKRVESKYGPPCPPCPAPEFLGGPSVFLFPPKPKDTLMISRTPEVTCVVVDVSQEDPEVQFNWYVDGVEVHNAKTKPREEQFNSTYRVVSVLTVLHQDWLNGKEYKCKVSNKGLPSSIEKTISKAKGQPREPQVYTLPPSQEEMTKNQVSLTCLVKGFYPSDIAVEWESNGQPENNYKTTPPVLDSDGSFFLYSRLTVDKSRWQEGNVFSCSVMHEALHNHYTQKSLSLSPGK

SEQ ID NO: 81 - skipped

SEQ ID NO: 82 - protein, 21 aa, Homo sapiens
DPGMYYWYYSGSAYEGYGLDY

SEQ ID NO: 83 - protein, 11 aa, Homo sapiens
QQRSRVYSLVT

SEQ ID NO: 84 - protein, 11 aa, Homo sapiens
QQMDRFYSLIT

SEQ ID NO: 85 - protein, 11 aa, Homo sapiens
QQYCRKSSLFT

SEQ ID NO: 86 - protein, 11 aa, Homo sapiens
QQQQRTSYLIT

SEQ ID NO: 87 - protein, 11 aa, Homo sapiens
QQRSRYYSLIT

SEQ ID NO: 88 - protein, 11 aa, Homo sapiens
QQSNRSYPPLT

SEQ ID NO: 89 - protein, 11 aa, Homo sapiens
QQIGRRSSLIT

SEQ ID NO: 90 - protein, 11 aa, Homo sapiens
QQQQRYSYLIT

SEQ ID NO: 91 - protein, 11 aa, Homo sapiens
QQSSRNSKLIT

SEQ ID NO: 92 - protein, 11 aa, Homo sapiens
QQWMRSSSLFT

SEQ ID NO: 93 - protein, 9 aa, Homo sapiens
  SITE 4: note = MISC_FEATURE - X may be S or T
  SITE 5: note = MISC_FEATURE - X may be S, G, or A
  SITE 6: note = MISC_FEATURE - X may be T, N, or S
  SITE 7: note = MISC_FEATURE - X may be D or S
FTFXXXXIH

SEQ ID NO: 94 - protein, 9 aa, Homo sapiens
  SITE 4: note = MISC_FEATURE - X may be S or T
  SITE 5: note = MISC_FEATURE - X may be S or A
  SITE 6: note = MISC_FEATURE - X may be N or S
  SITE 7: note = MISC_FEATURE - X may be D or S
FTFXXXXIH